European Patent Application EP 4 506 363 A1, published February 12, 2025. Title: 针对c-Met的单克隆抗体以及双特异性抗体. Applicant: 普米斯生物技术（珠海）有限公司. The sequence listing filed with the application follows.

SEQUENCE LISTING (53 sequences)

SEQ ID NO: 1 - protein, 125 aa, synthetic construct [sequence omitted]

SEQ ID NO: 2 - protein, 455 aa, synthetic construct
QVQLVESGGGVVQPGRSLRLSCAASGFTFSTYGMHWVRQAPGKGLEWVAVIWDDGSYKYYGDSVKGRFTISRDNSKNTLYLQMNSLRAEDTAVYYCARDGITMVRGVMKDYFDYWGQGTLVTVSSASTKGPSVFPLAPSSKSTSGGTAALGCLVKDYFPEPVTVSWNSGALTSGVHTFPAVLQSSGLYSLSSVVTVPSSSLGTQTYICNVNHKPSNTKVDKKVEPKSCDKTHTCPPCPAPELLGGPSVFLFPPKPKDTLMISRTPEVTCVVVDVSHEDPEVKFNWYVDGVEVHNAKTKPREEQYNSTYRVVSVLTVLHQDWLNGKEYKCKVSNKALPAPIEKTISKAKGQPREPQVYTEPPSRDELTKNQVSLTCLVKGFYPSDIAVEWESNGQPENNYKTTPPVLDSDGSFFLLSVLTVDKSRWQQGNVFSCSVMHEALHNHYTQKSLSLSPGK

SEQ ID NO: 3 - protein, 107 aa, synthetic construct [sequence omitted]

SEQ ID NO: 4 - protein, 214 aa, synthetic construct
AIQLTQSPSSLSASVGDRVTITCRASQDISSALVWYQQKPGKAPKLLIYDASSLESGVPSRFSGSESGTDFTLTISSLQPEDFATYYCQQFNSYPLTFGGGTKVEIKRTVAAPSVFIFPPSDEQLKSGTASVVCLLNNFYPREAKVQWKVDNALQSGNSQESVTEQDSKDSTYSLSSTLTLSKADYEKHKVYACEVTHQGLSSPVTKSFNRGEC

SEQ ID NO: 5 - protein, 119 aa, synthetic construct
QVQLVQSGAEVKKPGASVKVSCETSGYTFTSYGISWVRQAPGHGLEWMGWISAYNGYTNYAQKLQGRVTMTTDTSTSTAYMELRSLRSDDTAVYYCARDLRGTNYFDYWGQGTLVTVSS

SEQ ID NO: 6 - protein, 449 aa, synthetic construct
QVQLVQSGAEVKKPGASVKVSCETSGYTFTSYGISWVRQAPGHGLEWMGWISAYNGYTNYAQKLQGRVTMTTDTSTSTAYMELRSLRSDDTAVYYCARDLRGTNYFDYWGQGTLVTVSSASTKGPSVFPLAPSSKSTSGGTAALGCLVKDYFPEPVTVSWNSGALTSGVHTFPAVLQSSGLYSLSSVVTVPSSSLGTQTYICNVNHKPSNTKVDKKVEPKSCDKTHTCPPCPAPELLGGPSVFLFPPKPKDTLMISRTPEVTCVVVDVSHEDPEVKFNWYVDGVEVHNAKTKPREEQYNSTYRVVSVLTVLHQDWLNGKEYKCKVSNKALPAPIEKTISKAKGQPREPQVYTLPPSRDELTKNQVSLLCLVKGFYPSDIAVEWESNGQPENNYKTTPPVLRSDGSFFLYSKLTVDKSRWQQGNVFSCSVMHEALHNHYTQKSLSLSPGK

SEQ ID NO: 7 - protein, 107 aa, synthetic construct
DIQMTQSPSSVSASVGDRVTITCRASQGISNWLAWFQHKPGKAPKLLIYAASSLLSGVPSRFSGSGSGTDFTLTISSLQPEDFATYYCQQANSFPITFGQGTRLEIK

SEQ ID NO: 8 - protein, 214 aa, synthetic construct
DIQMTQSPSSVSASVGDRVTITCRASQGISNWLAWFQHKPGKAPKLLIYAASSLLSGVPSRFSGSGSGTDFTLTISSLQPEDFATYYCQQANSFPITFGQGTRLEIKRTVAAPSVFIFPPSDEQLKSGTASVVCLLNNFYPREAKVQWKVDNALQSGNSQESVTEQDSKDSTYSLSSTLTLSKADYEKHKVYACEVTHQGLSSPVTKSFNRGEC

SEQ ID NO: 9 - protein, 118 aa, synthetic construct
EVQLQESGPGLVKPSETLSLTCTVSGGSVTSVNYYWKWIRQPPGKGLEWIGYISYSGNTNYNPSLKSRVTISVDTSKNQFSLKLSSVTAADTAVYYCVRAPYYYMDVWSKGTTVTVSS

SEQ ID NO: 10 - protein, 447 aa, synthetic construct
EVQLQESGPGLVKPSETLSLTCTVSGGSVTSVNYYWKWIRQPPGKGLEWIGYISYSGNTNYNPSLKSRVTISVDTSKNQFSLKLSSVTAADTAVYYCVRAPYYYMDVWSKGTTVTVSSASTKGPSVFPLAPSSKSTSGGTAALGCLVKDYFPEPVTVSWNSGALTSGVHTFPAVLQSSGLYSLSSVVTVPSSSLGTQTYICNVNHKPSNTKVDKKVEPKSCDKTHTCPPCPAPELLGGPSVFLFPPKPKDTLMISRTPEVTCVVVDVSHEDPEVKFNWYVDGVEVHNAKTKPREEQYNSTYRVVSVLTVLHQDWLNGKEYKCKVSNKALPAPIEKTISKAKGQPREPQVYTLPPSRDELTKNQVSLLCLVKGFYPSDIAVEWESNGQPENNYKTTPPVLRSDGSFFLYSKLTVDKSRWQQGNVFSCSVMHEALHNHYTQKSLSLSPG

SEQ ID NO: 11 - protein, 107 aa, synthetic construct
DIVMTQSPSSVSASVGDRVTITCRASQGISSWLAWYQQKPGKAPKLLIYAVSSLQSGVPSRFSGSGSGTDFTLTISSLQPEDFATYFCQQANSFPLTFGGGTKVEIK

SEQ ID NO: 12 - protein, 214 aa, synthetic construct
DIVMTQSPSSVSASVGDRVTITCRASQGISSWLAWYQQKPGKAPKLLIYAVSSLQSGVPSRFSGSGSGTDFTLTISSLQPEDFATYFCQQANSFPLTFGGGTKVEIKRTVAAPSVFIFPPSDEQLKSGTASVVCLLNNFYPREAKVQWKVDNALQSGNSQESVTEQDSKDSTYSLSSTLTLSKADYEKHKVYACEVTHQGLSSPVTKSFNRGEC

SEQ ID NO: 13 - protein, 118 aa, synthetic construct
ELQLQESGPGLVKPSETLSLTCTVSGGSISSSSYYWGWIRQSPGKGLEWIGSRYYSGNTYYNPSLKSRVTMSVDTSKNQFSLKLRSVTAADTAVYYCARQVYDYWRDWGQGALVTVSS

SEQ ID NO: 14 - protein, 447 aa, synthetic construct
ELQLQESGPGLVKPSETLSLTCTVSGGSISSSSYYWGWIRQSPGKGLEWIGSRYYSGNTYYNPSLKSRVTMSVDTSKNQFSLKLRSVTAADTAVYYCARQVYDYWRDWGQGALVTVSSASTKGPSVFPLAPSSKSTSGGTAALGCLVKDYFPEPVTVSWNSGALTSGVHTFPAVLQSSGLYSLSSVVTVPSSSLGTQTYICNVNHKPSNTKVDKKVEPKSCDKTHTCPPCPAPELLGGPSVFLFPPKPKDTLMISRTPEVTCVVVDVSHEDPEVKFNWYVDGVEVHNAKTKPREEQYNSTYRVVSVLTVLHQDWLNGKEYKCKVSNKALPAPIEKTISKAKGQPREPQVYTLPPSRDELTKNQVSLLCLVKGFYPSDIAVEWESNGQPENNYKTTPPVLRSDGSFFLYSKLTVDKSRWQQGNVFSCSVMHEALHNHYTQKSLSLSPG

SEQ ID NO: 15 - protein, 107 aa, synthetic construct
DIVMTQSPSSVSASVGDRVTITCRASQGISSWLAWYQQKPGKAPNLLIYAASNLPSGVPSRFSGSGSGTVFTLTISSLQPEDFATYYCQQSNSFPLTFGGGTKVEIK

SEQ ID NO: 16 - protein, 214 aa, synthetic construct
DIVMTQSPSSVSASVGDRVTITCRASQGISSWLAWYQQKPGKAPNLLIYAASNLPSGVPSRFSGSGSGTVFTLTISSLQPEDFATYYCQQSNSFPLTFGGGTKVEIKRTVAAPSVFIFPPSDEQLKSGTASVVCLLNNFYPREAKVQWKVDNALQSGNSQESVTEQDSKDSTYSLSSTLTLSKADYEKHKVYACEVTHQGLSSPVTKSFNRGEC

SEQ ID NO: 17 - protein, 329 aa, synthetic construct
ASTKGPSVFPLAPSSKSTSGGTAALGCLVKDYFPEPVTVSWNSGALTSGVHTFPAVLQSSGLYSLSSVVTVPSSSLGTQTYICNVNHKPSNTKVDKKVEPKSCDKTHTCPPCPAPEAAGGPSVFLFPPKPKDTLMISRTPEVTCVVVDVSHEDPEVKFNWYVDGVEVHNAKTKPREEQYNSTYRVVSVLTVLHQDWLNGKEYKCKVSNKALPAPIEKTISKAKGQPREPQVYTLPPCRDELTKNQVSLWCLVKGFYPSDIAVEWESNGQPENNYKTTPPVLDSDGSFFLYSKLTVDKSRWQQGNVFSCSVMHEALHNHYTQKSLSLSPG

SEQ ID NO: 18 - protein, 226 aa, synthetic construct
DKTHTCPPCPAPEAAGGPSVFLFPPKPKDTLMISRTPEVTCVVVDVSHEDPEVKFNWYVDGVEVHNAKTKPREEQYNSTYRVVSVLTVLHQDWLNGKEYKCKVSNKALPAPIEKTISKAKGQPREPQVCTLPPSRDELTKNQVSLSCAVKGFYPSDIAVEWESNGQPENNYKTTPPVLDSDGSFFLVSKLTVDKSRWQQGNVFSCSVMHEALHNHYTQKSLSLSPG

SEQ ID NO: 19 - protein, 329 aa, synthetic construct
ASTKGPSVFPLAPSSKSTSGGTAALGCQVEDYFPEPVTVSWNSGALTSGVHTFPAVLQSSGLYELSSVVTVPSSSLGTQTYICNVNHKPSNTKVDKKVEPKSCDKTHTCPPCPAPELLGGPSVFLFPPKPKDTLMISRTPEVTCVVVDVSHEDPEVKFNWYVDGVEVHNAKTKPREEQYNSTYRVVSVLTVLHQDWLNGKEYKCKVSNKALPAPIEKTISKAKGQPREPQVYTLPPCRDELTKNQVSLWCLVKGFYPSDIAVEWESNGQPENNYKTTPPVLDSDGSFFLYSKLTVDKSRWQQGNVFSCSVMHEALHNHYTQKSLSLSPG

SEQ ID NO: 20 - protein, 329 aa, synthetic construct
ASTKGPSVFPRAPSSKSTSGGTAALGCLVRDYFPEPVTVSWNSGALTSGVHTFPAVLQSSGLYSLSSVVTVPSSSLGTQTYICNVNHKPSNTKVDKKVEPKSCDKTHTCPPCPAPELLGGPSVFLFPPKPKDTLMISRTPEVTCVVVDVSHEDPEVKFNWYVDGVEVHNAKTKPREEQYNSTYRVVSVLTVLHQDWLNGKEYKCKVSNKALPAPIEKTISKAKGQPREPQVCTLPPSRDELTKNQVSLSCAVKGFYPSDIAVEWESNGQPENNYKTTPPVLDSDGSFFLVSKLTVDKSRWQQGNVFSCSVMHEALHNHYTQKSLSLSPG

SEQ ID NO: 21 - protein, 107 aa, synthetic construct
RTVAAPSVFIFPPSDEQLKSGRASVVCLLNNFYPREAKVQWKVDNALQSGNSQESVTEQDSKDSTYSLSSRLQLSKADYEKHKVYACEVTHQGLSSPVTKSFNRGEC

SEQ ID NO: 22 - protein, 107 aa, synthetic construct
RTVAAPSVFIFPPSDEELKSGTASVQCLLNNFYPREAKVQWKVDNALQSGNSQESVTEQDSKDSTYSLSSELTLSKADYEKHKVYACEVTHQGLSSPVTKSFNRGEC

SEQ ID NO: 23 - protein, 447 aa, synthetic construct
EVQLQESGPGLVKPSETLSLTCTVSGGSVTSVNYYWKWIRQPPGKGLEWIGYISYSGNTNYNPSLKSRVTISVDTSKNQFSLKLSSVTAADTAVYYCVRAPYYYMDVWSKGTTVTVSSASTKGPSVFPLAPSSKSTSGGTAALGCQVEDYFPEPVTVSWNSGALTSGVHTFPAVLQSSGLYELSSVVTVPSSSLGTQTYICNVNHKPSNTKVDKKVEPKSCDKTHTCPPCPAPELLGGPSVFLFPPKPKDTLMISRTPEVTCVVVDVSHEDPEVKFNWYVDGVEVHNAKTKPREEQYNSTYRVVSVLTVLHQDWLNGKEYKCKVSNKALPAPIEKTISKAKGQPREPQVYTLPPCRDELTKNQVSLWCLVKGFYPSDIAVEWESNGQPENNYKTTPPVLDSDGSFFLYSKLTVDKSRWQQGNVFSCSVMHEALHNHYTQKSLSLSPG

SEQ ID NO: 24 - protein, 214 aa, synthetic construct
DIVMTQSPSSVSASVGDRVTITCRASQGISSWLAWYQQKPGKAPKLLIYAVSSLQSGVPSRFSGSGSGTDFTLTISSLQPEDFATYFCQQANSFPLTFGGGTKVEIKRTVAAPSVFIFPPSDEQLKSGRASVVCLLNNFYPREAKVQWKVDNALQSGNSQESVTEQDSKDSTYSLSSRLQLSKADYEKHKVYACEVTHQGLSSPVTKSFNRGEC

SEQ ID NO: 25 - protein, 454 aa, synthetic construct
EVQLVESGGGVVQPGRSLRLSCAASGFTFSTYGMHWVRQAPGKGLEWVAVIWDDGSYKYYGDSVKGRFTISRDNSKNTLYLQMNSLRAEDTAVYYCARDGITMVRGVMKDYFDYWGQGTLVTVSSASTKGPSVFPRAPSSKSTSGGTAALGCLVRDYFPEPVTVSWNSGALTSGVHTFPAVLQSSGLYSLSSVVTVPSSSLGTQTYICNVNHKPSNTKVDKKVEPKSCDKTHTCPPCPAPELLGGPSVFLFPPKPKDTLMISRTPEVTCVVVDVSHEDPEVKFNWYVDGVEVHNAKTKPREEQYNSTYRVVSVLTVLHQDWLNGKEYKCKVSNKALPAPIEKTISKAKGQPREPQVCTLPPSRDELTKNQVSLSCAVKGFYPSDIAVEWESNGQPENNYKTTPPVLDSDGSFFLVSKLTVDKSRWQQGNVFSCSVMHEALHNHYTQKSLSLSPG

SEQ ID NO: 26 - protein, 214 aa, synthetic construct
DIQLTQSPSSLSASVGDRVTITCRASQDISSALVWYQQKPGKAPKLLIYDASSLESGVPSRFSGSESGTDFTLTISSLQPEDFATYYCQQFNSYPLTFGGGTKVEIKRTVAAPSVFIFPPSDEELKSGTASVQCLLNNFYPREAKVQWKVDNALQSGNSQESVTEQDSKDSTYSLSSELTLSKADYEKHKVYACEVTHQGLSSPVTKSFNRGEC

SEQ ID NO: 27 - protein, 10 aa, synthetic construct
GGSVTSVNYY

SEQ ID NO: 28 - protein, 7 aa, synthetic construct
ISYSGNT

SEQ ID NO: 29 - protein, 10 aa, synthetic construct
VRAPYYYMDV

SEQ ID NO: 30 - protein, 6 aa, synthetic construct
QGISSW

SEQ ID NO: 31 - skipped

SEQ ID NO: 32 - protein, 9 aa, synthetic construct
QQANSFPLT

SEQ ID NO: 33 - protein, 10 aa, synthetic construct
GGSISSSSYY

SEQ ID NO: 34 - protein, 7 aa, synthetic construct
RYYSGNT

SEQ ID NO: 35 - protein, 10 aa, synthetic construct
ARQVYDYWRD

SEQ ID NO: 36 - protein, 6 aa, synthetic construct
QGISSW

SEQ ID NO: 37 - skipped

SEQ ID NO: 38 - protein, 9 aa, synthetic construct
QQSNSFPLT

SEQ ID NO: 39 - protein, 330 aa, synthetic construct
ASTKGPSVFPLAPSSKSTSGGTAALGCLVKDYFPEPVTVSWNSGALTSGVHTFPAVLQSSGLYSLSSVVTVPSSSLGTQTYICNVNHKPSNTKVDKKVEPKSCDKTHTCPPCPAPELLGGPSVFLFPPKPKDTLMISRTPEVTCVVVDVSHEDPEVKFNWYVDGVEVHNAKTKPREEQYNSTYRVVSVLTVLHQDWLNGKEYKCKVSNKALPAPIEKTISKAKGQPREPQVYTEPPSRDELTKNQVSLTCLVKGFYPSDIAVEWESNGQPENNYKTTPPVLDSDGSFFLLSVLTVDKSRWQQGNVFSCSVMHEALHNHYTQKSLSLSPGK

SEQ ID NO: 40 - protein, 329 aa, synthetic construct
ASTKGPSVFPLAPSSKSTSGGTAALGCLVKDYFPEPVTVSWNSGALTSGVHTFPAVLQSSGLYSLSSVVTVPSSSLGTQTYICNVNHKPSNTKVDKKVEPKSCDKTHTCPPCPAPELLGGPSVFLFPPKPKDTLMISRTPEVTCVVVDVSHEDPEVKFNWYVDGVEVHNAKTKPREEQYNSTYRVVSVLTVLHQDWLNGKEYKCKVSNKALPAPIEKTISKAKGQPREPQVYTLPPSRDELTKNQVSLLCLVKGFYPSDIAVEWESNGQPENNYKTTPPVLRSDGSFFLYSKLTVDKSRWQQGNVFSCSVMHEALHNHYTQKSLSLSPG

SEQ ID NO: 41 - protein, 107 aa, synthetic construct [sequence omitted]

SEQ ID NO: 42 - protein, 454 aa, synthetic construct
QVQLVESGGGVVQPGRSLRLSCAASGFTFSTYGMHWVRQAPGKGLEWVAVIWDDGSYKYYGDSVKGRFTISRDNSKNTLYLQMNSLRAEDTAVYYCARDGITMVRGVMKDYFDYWGQGTLVTVSSASTKGPSVFPLAPSSKSTSGGTAALGCLVKDYFPEPVTVSWNSGALTSGVHTFPAVLQSSGLYSLSSVVTVPSSSLGTQTYICNVNHKPSNTKVDKKVEPKSCDKTHTCPPCPAPEAAGGPSVFLFPPKPKDTLMISRTPEVTCVVVDVSHEDPEVKFNWYVDGVEVHNAKTKPREEQYNSTYRVVSVLTVLHQDWLNGKEYKCKVSNKALPAPIEKTISKAKGQPREPQVYTLPPCRDELTKNQVSLWCLVKGFYPSDIAVEWESNGQPENNYKTTPPVLDSDGSFFLYSKLTVDKSRWQQGNVFSCSVMHEALHNHYTQKSLSLSPG

SEQ ID NO: 43 - protein, 448 aa, synthetic construct
QVQLVQSGAEVKKPGASVKVSCETSGYTFTSYGISWVRQAPGHGLEWMGWISAYNGYTNYAQKLQGRVTMTTDTSTSTAYMELRSLRSDDTAVYYCARDLRGTNYFDYWGQGTLVTVSSASTKGPSVFPLAPSSKSTSGGTAALGCLVKDYFPEPVTVSWNSGALTSGVHTFPAVLQSSGLYSLSSVVTVPSSSLGTQTYICNVNHKPSNTKVDKKVEPKSCDKTHTCPPCPAPEAAGGPSVFLFPPKPKDTLMISRTPEVTCVVVDVSHEDPEVKFNWYVDGVEVHNAKTKPREEQYNSTYRVVSVLTVLHQDWLNGKEYKCKVSNKALPAPIEKTISKAKGQPREPQVYTLPPCRDELTKNQVSLWCLVKGFYPSDIAVEWESNGQPENNYKTTPPVLDSDGSFFLYSKLTVDKSRWQQGNVFSCSVMHEALHNHYTQKSLSLSPG

SEQ ID NO: 44 - protein, 447 aa, synthetic construct
EVQLQESGPGLVKPSETLSLTCTVSGGSVTSVNYYWKWIRQPPGKGLEWIGYISYSGNTNYNPSLKSRVTISVDTSKNQFSLKLSSVTAADTAVYYCVRAPYYYMDVWSKGTTVTVSSASTKGPSVFPLAPSSKSTSGGTAALGCLVKDYFPEPVTVSWNSGALTSGVHTFPAVLQSSGLYSLSSVVTVPSSSLGTQTYICNVNHKPSNTKVDKKVEPKSCDKTHTCPPCPAPEAAGGPSVFLFPPKPKDTLMISRTPEVTCVVVDVSHEDPEVKFNWYVDGVEVHNAKTKPREEQYNSTYRVVSVLTVLHQDWLNGKEYKCKVSNKALPAPIEKTISKAKGQPREPQVYTLPPCRDELTKNQVSLWCLVKGFYPSDIAVEWESNGQPENNYKTTPPVLDSDGSFFLYSKLTVDKSRWQQGNVFSCSVMHEALHNHYTQKSLSLSPG

SEQ ID NO: 45 - protein, 447 aa, synthetic construct
ELQLQESGPGLVKPSETLSLTCTVSGGSISSSSYYWGWIRQSPGKGLEWIGSRYYSGNTYYNPSLKSRVTMSVDTSKNQFSLKLRSVTAADTAVYYCARQVYDYWRDWGQGALVTVSSASTKGPSVFPLAPSSKSTSGGTAALGCLVKDYFPEPVTVSWNSGALTSGVHTFPAVLQSSGLYSLSSVVTVPSSSLGTQTYICNVNHKPSNTKVDKKVEPKSCDKTHTCPPCPAPEAAGGPSVFLFPPKPKDTLMISRTPEVTCVVVDVSHEDPEVKFNWYVDGVEVHNAKTKPREEQYNSTYRVVSVLTVLHQDWLNGKEYKCKVSNKALPAPIEKTISKAKGQPREPQVYTLPPCRDELTKNQVSLWCLVKGFYPSDIAVEWESNGQPENNYKTTPPVLDSDGSFFLYSKLTVDKSRWQQGNVFSCSVMHEALHNHYTQKSLSLSPG

SEQ ID NO: 46 - protein, 8 aa, synthetic construct
GFTFSTYG

SEQ ID NO: 47 - protein, 8 aa, synthetic construct
IWDDGSYK

SEQ ID NO: 48 - protein, 18 aa, synthetic construct
ARDGITMVRGVMKDYFDY

SEQ ID NO: 49 - protein, 6 aa, synthetic construct
QDISSA

SEQ ID NO: 50 - skipped

SEQ ID NO: 51 - protein, 9 aa, synthetic construct
QQFNSYPLT

SEQ ID NO: 52 - protein, 125 aa, synthetic construct
EVQLVESGGGVVQPGRSLRLSCAASGFTFSTYGMHWVRQAPGKGLEWVAVIWDDGSYKYYGDSVKGRFTISRDNSKNTLYLQMNSLRAEDTAVYYCARDGITMVRGVMKDYFDYWGQGTLVTVSS

SEQ ID NO: 53 - protein, 107 aa, synthetic construct
DIQLTQSPSSLSASVGDRVTITCRASQDISSALVWYQQKPGKAPKLLIYDASSLESGVPSRFSGSESGTDFTLTISSLQPEDFATYYCQQFNSYPLTFGGGTKVEIK